European Patent Application EP 4 772 534 A1, published July 8, 2026. Title: Fc variant. Applicant: Astellas Pharma Inc. The sequence listing filed with the application follows.

SEQUENCE LISTING (24 sequences)

SEQ ID NO: 1 - protein, 449 aa, Homo sapiens
QVQLVQSGAEVKKPGASVKVSCKASGYAFSSSWVNWVRQAPGQGLEWMGRIYPGDGDTDYNGKFKGRVTLTADKSTSTAYMELSSLRSEDTAVYYCARRRGYEAVFDYWGQGTLVTVSSASTKGPSVFPLAPSSKSTSGGTAALGCLVKDYFPEPVTVSWNSGALTSGVHTFPAVLQSSGLYSLSSVVTVPSSSLGTQTYICNVNHKPSNTKVDKKVEPKSCDKTHTCPPCPAPELLGGPSVFLFPPKPKDTLMISRTPEVTCVVVDVSHEDPEVKFNWYVDGVEVHNAKTKPREEQYNSTYRVVSVLTVLHQDWLNGKEYKCKVSNKALPAPIEKTISKAKGQPREPQVYTLPPSRDELTKNQVSLTCLVKGFYPSDIAVEWESNGQPENNYKTTPPVLDSDGSFFLYSKLTVDKSRWQQGNVFSCSVMHEALHNHYTQKSLSLSPGK

SEQ ID NO: 2 - DNA, 1347 bp, Homo sapiens
  source 1..1347: mol_type = other DNA
caggtgcagctggttcagtctggcgccgaagtgaagaaacctggcgcctctgtgaaggtgtcctgcaaggcttctggctacgccttctcctcctcctgggtcaactgggtccgacaggctcctggacaaggcctggaatggatgggcagaatctatcctggcgacggcgacaccgactacaacggcaagtttaagggcagagtgaccctgaccgccgacaagtctacctccaccgcctacatggaactgtccagcctgagatctgaggacaccgccgtgtactactgcgctcggagaagaggctacgaggccgtgtttgattattggggccagggcaccctggtcaccgtgtcctctgcttctaccaagggacccagcgtgttccctctggctcctagctctaagtccacctctggcggaacagctgctctgggctgtctggtcaaggactacttccctgagcctgtgaccgtgtcttggaactctggcgctctgacatccggcgtgcacacctttccagctgtgctgcaatcctccggcctgtactctctgtcctccgtcgtgaccgtgccttctagctctctgggcacccagacctacatctgcaatgtgaaccacaagccttccaacaccaaggtggacaagaaggtggaacccaagtcctgcgacaagacccacacctgtcctccatgtcctgctccagaactgctcggcggaccttccgtgtttctgttccctccaaagcctaaggacaccctgatgatctctcggacccctgaagtgacctgcgtggtggtggatgtgtctcacgaggacccagaagtgaagttcaattggtacgtggacggcgtggaagtgcacaacgccaagaccaagcctagagaggaacagtacaactccacctacagagtggtgtccgtgctgaccgtgctgcaccaggattggctgaacggcaaagagtacaagtgcaaggtgtccaacaaggccctgcctgctcctatcgaaaagaccatctccaaggccaagggccagcctagggaaccccaggtttacaccttgcctccatctcgggacgagctgaccaagaaccaggtgtccctgacctgtctcgtgaagggcttctacccctccgatatcgccgtggaatgggagtctaatggccagccagagaacaactacaagacaacccctcctgtgctggactccgacggctcattcttcctgtactccaagctgacagtggacaagtccagatggcagcagggcaacgtgttctcctgctccgtgatgcacgaggccctgcacaatcactacacacagaagtccctgtctctgtcccctggcaag

SEQ ID NO: 3 - protein, 218 aa, Homo sapiens
DIQLTQSPSSLSASVGDRVTITCRASESVDNYDISFLNWFQQKPGKAPKLLIYAASNQGSGVPSRFSGSGSGTDFTLTISSLQPEDFATYYCQQSKEVPYTFGGGTKVEIKRTVAAPSVFIFPPSDEQLKSGTASVVCLLNNFYPREAKVQWKVDNALQSGNSQESVTEQDSKDSTYSLSSTLTLSKADYEKHKVYACEVTHQGLSSPVTKSFNRGEC

SEQ ID NO: 4 - DNA, 654 bp, Homo sapiens
  source 1..654: mol_type = other DNA
gacatccagctgacccagagcccttccagcctgtctgcttccgtgggcgacagagtgaccatcacctgtcgggcctccgagtccgtggacaactacgatatctccttcctgaactggttccagcagaagcccggcaaggcccccaagctgctgatctacgccgcctccaatcagggctccggcgtgccctctagattctccggctctggctctggcaccgactttaccctgaccatctccagcctgcagcccgaggacttcgccacctactactgccagcagtccaaagaggtgccctacaccttcggcggaggcaccaaggtggaaatcaagcggaccgtggccgctccctccgtgttcatcttcccaccttccgacgagcagctgaagtccggcaccgcttctgtcgtgtgcctgctgaacaacttctacccccgcgaggccaaggtgcagtggaaggtggacaacgccctgcagtccggcaactcccaggaatccgtgaccgagcaggactccaaggacagcacctactccctgtcctccaccctgaccctgtccaaggccgactacgagaagcacaaggtgtacgcctgcgaagtgacccaccagggcctgtctagccccgtgaccaagtctttcaaccggggcgagtgc

SEQ ID NO: 5 - protein, 448 aa, Homo sapiens
QVQLVQSGAEVKKPGASVKVSCKASGYAFSSSWVNWVRQAPGQGLEWMGRIYPGDGDTDYNGKFKGRVTLTADKSTSTAYMELSSLRSEDTAVYYCARRRGYEAVFDYWGQGTLVTVSSASTKGPSVFPLAPSSKSTSGGTAALGCLVKDYFPEPVTVSWNSGALTSGVHTFPAVLQSSGLYSLSSVVTVPSSSLGTQTYICNVNHKPSNTKVDKKVEPKSCDKTHTCPPCPAPELLGGPSVFLFPPKPKDTLMISRTPEVTCVVVDVSHEDPEVKFNWYVDGVEVHNAKTKPREQYNSTYRVVSVLTVLHQDWLNGKEYKCKVSNKALPAPIEKTISKAKGQPREPQVYTLPPSRDELTKNQVSLTCLVKGFYPSDIAVEWESNGQPENNYKTTPPVLDSDGSFFLYSKLTVDKSRWQQGNVFSCSVMHEALHNHYTQKSLSLSPGK

SEQ ID NO: 6 - DNA, 1344 bp, Homo sapiens
  source 1..1344: mol_type = other DNA
caggtgcagctggttcagtctggcgccgaagtgaagaaacctggcgcctctgtgaaggtgtcctgcaaggcttctggctacgccttctcctcctcctgggtcaactgggtccgacaggctcctggacaaggcctggaatggatgggcagaatctatcctggcgacggcgacaccgactacaacggcaagtttaagggcagagtgaccctgaccgccgacaagtctacctccaccgcctacatggaactgtccagcctgagatctgaggacaccgccgtgtactactgcgctcggagaagaggctacgaggccgtgtttgattattggggccagggcaccctggtcaccgtgtcctctgcttctaccaagggacccagcgtgttccctctggctcctagctctaagtccacctctggcggaacagctgctctgggctgtctggtcaaggactacttccctgagcctgtgaccgtgtcttggaactctggcgctctgacatccggcgtgcacacctttccagctgtgctgcaatcctccggcctgtactctctgtcctccgtcgtgaccgtgccttctagctctctgggcacccagacctacatctgcaatgtgaaccacaagccttccaacaccaaggtggacaagaaggtggaacccaagtcctgcgacaagacccacacctgtcctccatgtcctgctccagaactgctcggcggaccttccgtgtttctgttccctccaaagcctaaggacaccctgatgatctctcggacccctgaagtgacctgcgtggtggtggatgtgtctcacgaggacccagaagtgaagttcaattggtacgtggacggcgtggaagtgcacaacgccaagaccaagcctagagagcagtacaactccacctacagagtggtgtccgtgctgaccgtgctgcaccaggattggctgaacggcaaagagtacaagtgcaaggtgtccaacaaggccctgcctgctcctatcgaaaagaccatctccaaggccaagggccagcctagggaaccccaggtttacaccttgcctccatctcgggacgagctgaccaagaaccaggtgtccctgacctgtctcgtgaagggcttctacccctccgatatcgccgtggaatgggagtctaatggccagccagagaacaactacaagacaacccctcctgtgctggactccgacggctcattcttcctgtactccaagctgacagtggacaagtccagatggcagcagggcaacgtgttctcctgctccgtgatgcacgaggccctgcacaatcactacacacagaagtccctgtctctgtcccctggcaag

SEQ ID NO: 7 - protein, 448 aa, Homo sapiens
QVQLVQSGAEVKKPGASVKVSCKASGYAFSSSWVNWVRQAPGQGLEWMGRIYPGDGDTDYNGKFKGRVTLTADKSTSTAYMELSSLRSEDTAVYYCARRRGYEAVFDYWGQGTLVTVSSASTKGPSVFPLAPSSKSTSGGTAALGCLVKDYFPEPVTVSWNSGALTSGVHTFPAVLQSSGLYSLSSVVTVPSSSLGTQTYICNVNHKPSNTKVDKKVEPKSCDKTHTCPPCPAPEAAGGPSVFLFPPKPKDTLMISRTPEVTCVVVDVSHEDPEVKFNWYVDGVEVHNAKTKPREQYNSTYRVVSVLTVLHQDWLNGKEYKCKVSNKALPAPIEKTISKAKGQPREPQVYTLPPSRDELTKNQVSLTCLVKGFYPSDIAVEWESNGQPENNYKTTPPVLDSDGSFFLYSKLTVDKSRWQQGNVFSCSVMHEALHNHYTQKSLSLSPGK

SEQ ID NO: 8 - DNA, 1344 bp, Homo sapiens
  source 1..1344: mol_type = other DNA
caggtgcagctggttcagtctggcgccgaagtgaagaaacctggcgcctctgtgaaggtgtcctgcaaggcttctggctacgccttctcctcctcctgggtcaactgggtccgacaggctcctggacaaggcctggaatggatgggcagaatctatcctggcgacggcgacaccgactacaacggcaagtttaagggcagagtgaccctgaccgccgacaagtctacctccaccgcctacatggaactgtccagcctgagatctgaggacaccgccgtgtactactgcgctcggagaagaggctacgaggccgtgtttgattattggggccagggcaccctggtcaccgtgtcctctgcttctaccaagggacccagcgtgttccctctggctcctagctctaagtccacctctggcggaacagctgctctgggctgtctggtcaaggactacttccctgagcctgtgaccgtgtcttggaactctggcgctctgacatccggcgtgcacacctttccagctgtgctgcaatcctccggcctgtactctctgtcctccgtcgtgaccgtgccttctagctctctgggcacccagacctacatctgcaatgtgaaccacaagccttccaacaccaaggtggacaagaaggtggaacccaagtcctgcgacaagacccacacctgtcctccatgtcctgctccagaagctgctggcggcccttccgtgtttctgttccctccaaagcctaaggacaccctgatgatctctcggacccctgaagtgacctgcgtggtggtggatgtgtctcacgaggacccagaagtgaagttcaattggtacgtggacggcgtggaagtgcacaacgccaagaccaagcctagagagcagtacaactccacctacagagtggtgtccgtgctgaccgtgctgcaccaggattggctgaacggcaaagagtacaagtgcaaggtgtccaacaaggccctgcctgctcctatcgaaaagaccatctccaaggccaagggccagcctagggaaccccaggtttacaccttgcctccatctcgggacgagctgaccaagaaccaggtgtccctgacctgtctcgtgaagggcttctacccctccgatatcgccgtggaatgggagtctaatggccagccagagaacaactacaagacaacccctcctgtgctggactccgacggctcattcttcctgtactccaagctgacagtggacaagtccagatggcagcagggcaacgtgttctcctgctccgtgatgcacgaggccctgcacaatcactacacacagaagtccctgtctctgtcccctggcaag

SEQ ID NO: 9 - protein, 447 aa, Homo sapiens
EVQLVESGGGLVQPGGSLRLSCAASGFTFSLFTMSWVRQAPGKGLEWVSAISGSGGSTYYADSVKGRFTISRDNSKNTLYLQMNSLRAEDTAVYYCAKSTHLYLFDYWGQGTLVTVSSASTKGPSVFPLAPSSKSTSGGTAALGCLVKDYFPEPVTVSWNSGALTSGVHTFPAVLQSSGLYSLSSVVTVPSSSLGTQTYICNVNHKPSNTKVDKKVEPKSCDKTHTCPPCPAPELLGGPSVFLFPPKPKDTLMISRTPEVTCVVVDVSHEDPEVKFNWYVDGVEVHNAKTKPREQYNSTYRVVSVLTVLHQDWLNGKEYKCKVSNKALPAPIEKTISKAKGQPREPQVYTLPPSRDELTKNQVSLTCLVKGFYPSDIAVEWESNGQPENNYKTTPPVLDSDGSFFLYSKLTVDKSRWQQGNVFSCSVMHEALHNHYTQKSLSLSPGK

SEQ ID NO: 10 - DNA, 1341 bp, Homo sapiens
  source 1..1341: mol_type = other DNA
gaagttcaactcgtggaatccggcggcggcctggttcagccaggtggcagcctccgactctcatgtgcagccagtggattcacattcagtcttttcaccatgtcttgggttaggcaggctcccggaaagggcctggaatgggtttcagcaatcagcggatcaggtggcagtacctactacgctgatagcgtcaagggccgtttcacaatcagtcgggacaatagcaagaatactctttatcttcaaatgaatagcctgcgcgcagaagatacagccgtctactattgcgcaaagtcaactcatctctacctctttgattattggggacagggcacccttgtgacagtaagctcagcctccacaaaaggtccttctgtgtttcctctcgctccatcttccaaatcaacctcaggtggcacagccgcccttgggtgcctcgttaaagattacttccctgaacctgttaccgtcagctggaacagcggagccctgacctccggagtccacactttcccagctgttctgcagagcagtggcctctactcactcagcagtgttgtgactgtcccttcaagttctttgggtacacaaacttatatctgcaacgttaaccacaaaccatccaacaccaaagtcgataagaaggtcgagcctaagtcctgcgacaaaactcatacttgcccaccctgccccgcaccagagctcttgggaggtccaagcgtctttctcttccctcctaaacccaaggatacacttatgatatcaagaacccctgaggtcacatgtgtcgtcgtcgacgtatcacatgaggaccctgaggtgaaattcaattggtacgtagatggcgtcgaagtccataatgctaagaccaaacctcgagaacagtataacagtacttaccgagtagtttcagtcttgactgtgttgcaccaggactggctcaacgggaaggaatacaaatgcaaagtttctaacaaggctttgcctgctccaattgagaaaactattagcaaggccaagggtcagccccgtgagccacaagtatatactcttcctccttcaagggacgaattgaccaagaaccaggtttccttgacttgcttggttaaaggattctaccccagtgacatcgcagtggaatgggaaagtaacgggcagcctgagaataattacaagactactcctcctgtgcttgattcagatggaagtttcttcctttacagtaagttgactgtagacaaaagtcgatggcaacaagggaatgtgttttcttgttctgtgatgcatgaggcattgcataaccattatacacagaaatccctgtcattgtccccaggtaaa

SEQ ID NO: 11 - protein, 215 aa, Homo sapiens
EIVLTQSPGTLSLSPGEKATLSCRASQSVSMPFLAWYQQKPGQAPRLLIYGASSRATGIPDRFSGSGSGTDFTLTISRLEPEDFAVYYCQQMRGRPPTFGQGTKVEIKRTVAAPSVFIFPPSDEQLKSGTASVVCLLNNFYPREAKVQWKVDNALQSGNSQESVTEQDSKDSTYSLSSTLTLSKADYEKHKVYACEVTHQGLSSPVTKSFNRGEC

SEQ ID NO: 12 - DNA, 645 bp, Homo sapiens
  source 1..645: mol_type = other DNA
gaaatagtattgacccagtcacctggtacactgtcactgtctccaggagaaaaggcaaccttgtcatgccgggcaagccagtctgtgtccatgcctttcttggcatggtaccagcagaagccaggtcaagctcccaggctgcttatctatggagctagctctagggctaccggtattcctgaccggttcagcggctcaggctctgggaccgatttcacactcaccattagcagactggaacctgaagactttgctgtctactactgccagcagatgcgaggaagacctcccaccttcggtcagggtactaaagtggagataaagagaaccgtcgctgctccctctgtattcatatttcctccaagtgatgaacagctgaagtccggcactgcctctgtggtttgcctgctcaacaacttttacccacgcgaggccaaggtgcagtggaaggtcgacaatgctctgcagagtggaaattcacaggaaagcgtgacagaacaagattccaaggactccacatatagccttagtagtactctgactctgtccaaagccgattatgagaaacataaagtatatgcctgtgaggttactcaccaggggctgtccagtcccgtgacaaaatcatttaaccgcggcgagtgc

SEQ ID NO: 13 - protein, 447 aa, Homo sapiens
EVQLVESGGGLVQPGGSLRLSCAASGFTFSLFTMSWVRQAPGKGLEWVSAISGSGGSTYYADSVKGRFTISRDNSKNTLYLQMNSLRAEDTAVYYCAKSTHLYLFDYWGQGTLVTVSSASTKGPSVFPLAPSSKSTSGGTAALGCLVKDYFPEPVTVSWNSGALTSGVHTFPAVLQSSGLYSLSSVVTVPSSSLGTQTYICNVNHKPSNTKVDKKVEPKSCDKTHTCPPCPAPEAAGGPSVFLFPPKPKDTLMISRTPEVTCVVVDVSHEDPEVKFNWYVDGVEVHNAKTKPREQYNSTYRVVSVLTVLHQDWLNGKEYKCKVSNKALPAPIEKTISKAKGQPREPQVYTLPPSRDELTKNQVSLTCLVKGFYPSDIAVEWESNGQPENNYKTTPPVLDSDGSFFLYSKLTVDKSRWQQGNVFSCSVMHEALHNHYTQKSLSLSPGK

SEQ ID NO: 14 - DNA, 1341 bp, Homo sapiens
  source 1..1341: mol_type = other DNA
gaagttcaactcgtggaatccggcggcggcctggttcagccaggtggcagcctccgactctcatgtgcagccagtggattcacattcagtcttttcaccatgtcttgggttaggcaggctcccggaaagggcctggaatgggtttcagcaatcagcggatcaggtggcagtacctactacgctgatagcgtcaagggccgtttcacaatcagtcgggacaatagcaagaatactctttatcttcaaatgaatagcctgcgcgcagaagatacagccgtctactattgcgcaaagtcaactcatctctacctctttgattattggggacagggcacccttgtgacagtaagctcagcttctaccaagggacccagcgtgttccctctggctcctagctctaagtccacctctggcggaacagctgctctgggctgtctggtcaaggactacttccctgagcctgtgaccgtgtcttggaactctggcgctctgacatccggcgtgcacacctttccagctgtgctgcaatcctccggcctgtactctctgtcctccgtcgtgaccgtgccttctagctctctgggcacccagacctacatctgcaatgtgaaccacaagccttccaacaccaaggtggacaagaaggtggaacccaagtcctgcgacaagacccacacctgtcctccatgtcctgctccagaagctgctggcggcccttccgtgtttctgttccctccaaagcctaaggacaccctgatgatctctcggacccctgaagtgacctgcgtggtggtggatgtgtctcacgaggacccagaagtgaagttcaattggtacgtggacggcgtggaagtgcacaacgccaagaccaagcctagagagcagtacaactccacctacagagtggtgtccgtgctgaccgtgctgcaccaggattggctgaacggcaaagagtacaagtgcaaggtgtccaacaaggccctgcctgctcctatcgaaaagaccatctccaaggccaagggccagcctagggaaccccaggtttacaccttgcctccatctcgggacgagctgaccaagaaccaggtgtccctgacctgtctcgtgaagggcttctacccctccgatatcgccgtggaatgggagtctaatggccagccagagaacaactacaagacaacccctcctgtgctggactccgacggctcattcttcctgtactccaagctgacagtggacaagtccagatggcagcagggcaacgtgttctcctgctccgtgatgcacgaggccctgcacaatcactacacacagaagtccctgtctctgtcccctggcaag

SEQ ID NO: 15 - protein, 448 aa, Homo sapiens
QVELVESGGGLVQPGGSLRLSCAASGFTFSLFTMSWVRQAPGKGLEWVSAISGSGGSTYYADSVKGRFTISRDNSKNTLYLQMNSLRAEDTAVYYCARSTHLYLFDYWGQGTLVTVSSASTKGPSVFPLAPSSKSTSGGTAALGCLVKDYFPEPVTVSWNSGALTSGVHTFPAVLQSSGLYSLSSVVTVPSSSLGTQTYICNVNHKPSNTKVDKKVEPKSCDKTHTCPPCPAPELLGGPSVFLFPPKPKDTLMISRTPEVTCVVVDVSHEDPEVKFNWYVDGVEVHNAKTKPREEQYNSTYRVVSVLTVLHQDWLNGKEYKCKVSNKALPAPIEKTISKAKGQPREPQVYTLPPSRDELTKNQVSLTCLVKGFYPSDIAVEWESNGQPENNYKTTPPVLDSDGSFFLYSKLTVDKSRWQQGNVFSCSVMHEALHNHYTQKSLSLSPGK

SEQ ID NO: 16 - DNA, 1344 bp, Homo sapiens
  source 1..1344: mol_type = other DNA
caggtggaactggtggaatctggcggcggattggttcagcctggcggatctctgagactgtcttgtgccgcctccggcttcaccttcagcctgttcacaatgtcctgggtccgacaggctcctggcaaaggactggaatgggtgtccgccatctctggcagcggcggctctacctactacgccgattctgtgaagggcagattcaccatcagccgggacaactccaagaacaccctgtacctgcagatgaactccctgagagccgaggacaccgccgtgtactactgtgccagaagcacccacctgtatctgttcgactattggggccagggcaccctggtcacagtgtcctctgcttctaccaagggacccagcgtgttccctctggctccttccagcaagtctacctctggcggaacagctgctctgggctgcctggtcaaggactactttcctgagcctgtgaccgtgtcctggaactctggcgctctgacatctggcgtgcacacctttccagctgtgctgcagtcctccggcctgtactctctgtcctctgtcgtgaccgtgccttccagctctctgggaacccagacctacatctgcaatgtgaaccacaagccttccaacaccaaggtggacaagaaggtggaacccaagtcctgcgacaagacccacacctgtcctccatgtcctgctccagaactgctcggcggaccttccgtgtttctgttccctccaaagcctaaggacaccctgatgatctctcggacccctgaagtgacctgcgtggtggtggatgtgtctcacgaggatcccgaagtgaagttcaattggtacgtggacggcgtggaagtgcacaacgccaagaccaagcctagagaggaacagtacaactccacctacagagtggtgtccgtgctgaccgtgctgcaccaggattggctgaacggcaaagagtacaagtgcaaggtgtccaacaaggccctgcctgctcctatcgaaaagaccatctccaaggccaagggccagcctagggaaccccaggtttacaccttgcctccatctcgggacgagctgaccaagaaccaggtgtccctgacctgtctcgtgaagggcttctacccctccgatatcgccgtggaatgggagtctaatggccagcctgagaacaactacaagacaacccctcctgtgctggactccgacggctcattcttcctgtactccaagctgacagtggacaagtccagatggcagcagggcaacgtgttctcctgctccgtgatgcacgaggccctgcacaatcactacacccagaagtccctgtctctgtcccctggcaaa

SEQ ID NO: 17 - protein, 215 aa, Homo sapiens
DIVLTQSPATLSLSPGERATLSCRASQSVSMPFLAWYQQKPGQAPRLLIYGASSRATGVPARFSGSGSGTDFTLTISSLEPEDFATYYCQQMRGRPPTFGQGTKVEIKRTVAAPSVFIFPPSDEQLKSGTASVVCLLNNFYPREAKVQWKVDNALQSGNSQESVTEQDSKDSTYSLSSTLTLSKADYEKHKVYACEVTHQGLSSPVTKSFNRGEC

SEQ ID NO: 18 - DNA, 645 bp, Homo sapiens
  source 1..645: mol_type = other DNA
gacatcgtgctgacccagtctccagccacactgtcactgtctccaggcgagagagctaccctgtcctgtagagcctctcagtccgtgtctatgcccttcctggcctggtatcagcagaagcctggacaggctccccggctgttgatctacggcgcttcttctagagctaccggcgtgcccgctagattctccggatctggctctggcaccgactttaccctgaccatcagctccctggaacctgaggacttcgccacctactactgccagcagatgagaggcagacctcctacctttggccagggcaccaaggtggaaatcaagcggaccgtggccgctccctccgtgttcatcttcccaccttccgacgagcagctgaagtccggcaccgcttctgtcgtgtgcctgctgaacaacttctacccccgcgaggccaaggtgcagtggaaggtggacaacgccctgcagtccggcaactcccaggaatccgtgaccgagcaggactccaaggacagcacctactccctgtcctccaccctgaccctgtccaaggccgactacgagaagcacaaggtgtacgcctgcgaagtgacccaccagggcctgtctagccccgtgaccaagtctttcaaccggggcgagtgc

SEQ ID NO: 19 - protein, 448 aa, Homo sapiens
QVELVESGGGLVQPGGSLRLSCAASGFTFSLFTMSWVRQAPGKGLEWVSAISGSGGSTYYADSVKGRFTISRDNSKNTLYLQMNSLRAEDTAVYYCARSTHLYLFDYWGQGTLVTVSSASTKGPSVFPLAPSSKSTSGGTAALGCLVKDYFPEPVTVSWNSGALTSGVHTFPAVLQSSGLYSLSSVVTVPSSSLGTQTYICNVNHKPSNTKVDKKVEPKSCDKTHTCPPCPAPEAAGGPSVFLFPPKPKDTLMISRTPEVTCVVVDVSHEDPEVKFNWYVDGVEVHNAKTKPREEQYNSTYRVVSVLTVLHQDWLNGKEYKCKVSNKALPAPIEKTISKAKGQPREPQVYTLPPSRDELTKNQVSLTCLVKGFYPSDIAVEWESNGQPENNYKTTPPVLDSDGSFFLYSKLTVDKSRWQQGNVFSCSVMHEALHNHYTQKSLSLSPGK

SEQ ID NO: 20 - DNA, 1344 bp, Homo sapiens
  source 1..1344: mol_type = other DNA
caggtggaactggtggaatctggcggcggattggttcagcctggcggatctctgagactgtcttgtgccgcctccggcttcaccttcagcctgttcacaatgtcctgggtccgacaggctcctggcaaaggactggaatgggtgtccgccatctctggcagcggcggctctacctactacgccgattctgtgaagggcagattcaccatcagccgggacaactccaagaacaccctgtacctgcagatgaactccctgagagccgaggacaccgccgtgtactactgtgccagaagcacccacctgtatctgttcgactattggggccagggcaccctggtcacagtgtcctctgcttctaccaagggacccagcgtgttccctctggctccttccagcaagtctacctctggcggaacagctgctctgggctgcctggtcaaggactactttcctgagcctgtgaccgtgtcctggaactctggcgctctgacatctggcgtgcacacctttccagctgtgctgcagtcctccggcctgtactctctgtcctctgtcgtgaccgtgccttccagctctctgggaacccagacctacatctgcaatgtgaaccacaagccttccaacaccaaggtggacaagaaggtggaacccaagtcctgcgacaagacccacacctgtcctccatgtcctgctccagaagctgctggcggcccttccgtgtttctgttccctccaaagcctaaggacaccctgatgatctctcggacccctgaagtgacctgcgtggtggtggatgtgtctcacgaggatcccgaagtgaagttcaattggtacgtggacggcgtggaagtgcacaacgccaagaccaagcctagagaggaacagtacaactccacctacagagtggtgtccgtgctgaccgtgctgcaccaggattggctgaacggcaaagagtacaagtgcaaggtgtccaacaaggccctgcctgctcctatcgaaaagaccatctccaaggccaagggccagcctagggaaccccaggtttacaccttgcctccatctcgggacgagctgaccaagaaccaggtgtccctgacctgtctcgtgaagggcttctacccctccgatatcgccgtggaatgggagtctaatggccagcctgagaacaactacaagacaacccctcctgtgctggactccgacggctcattcttcctgtactccaagctgacagtggacaagtccagatggcagcagggcaacgtgttctcctgctccgtgatgcacgaggccctgcacaatcactacacccagaagtccctgtctctgtcccctggcaaa

SEQ ID NO: 21 - protein, 447 aa, Homo sapiens
QVELVESGGGLVQPGGSLRLSCAASGFTFSLFTMSWVRQAPGKGLEWVSAISGSGGSTYYADSVKGRFTISRDNSKNTLYLQMNSLRAEDTAVYYCARSTHLYLFDYWGQGTLVTVSSASTKGPSVFPLAPSSKSTSGGTAALGCLVKDYFPEPVTVSWNSGALTSGVHTFPAVLQSSGLYSLSSVVTVPSSSLGTQTYICNVNHKPSNTKVDKKVEPKSCDKTHTCPPCPAPELLGGPSVFLFPPKPKDTLMISRTPEVTCVVVDVSHEDPEVKFNWYVDGVEVHNAKTKPREQYNSTYRVVSVLTVLHQDWLNGKEYKCKVSNKALPAPIEKTISKAKGQPREPQVYTLPPSRDELTKNQVSLTCLVKGFYPSDIAVEWESNGQPENNYKTTPPVLDSDGSFFLYSKLTVDKSRWQQGNVFSCSVMHEALHNHYTQKSLSLSPGK

SEQ ID NO: 22 - DNA, 1341 bp, Homo sapiens
  source 1..1341: mol_type = other DNA
caggtggaactggtggaatctggcggcggattggttcagcctggcggatctctgagactgtcttgtgccgcctccggcttcaccttcagcctgttcacaatgtcctgggtccgacaggctcctggcaaaggactggaatgggtgtccgccatctctggcagcggcggctctacctactacgccgattctgtgaagggcagattcaccatcagccgggacaactccaagaacaccctgtacctgcagatgaactccctgagagccgaggacaccgccgtgtactactgtgccagaagcacccacctgtatctgttcgactattggggccagggcaccctggtcacagtgtcctctgcttctaccaagggacccagcgtgttccctctggctccttccagcaagtctacctctggcggaacagctgctctgggctgcctggtcaaggactactttcctgagcctgtgaccgtgtcctggaactctggcgctctgacatctggcgtgcacacctttccagctgtgctgcagtcctccggcctgtactctctgtcctctgtcgtgaccgtgccttccagctctctgggaacccagacctacatctgcaatgtgaaccacaagccttccaacaccaaggtggacaagaaggtggaacccaagtcctgcgacaagacccacacctgtcctccatgtcctgctccagaactgctcggcggaccttccgtgtttctgttccctccaaagcctaaggacaccctgatgatctctcggacccctgaagtgacctgcgtggtggtggatgtgtctcacgaggatcccgaagtgaagttcaattggtacgtggacggcgtggaagtgcacaacgccaagaccaagcctagagagcagtacaactccacctacagagtggtgtccgtgctgaccgtgctgcaccaggattggctgaacggcaaagagtacaagtgcaaggtgtccaacaaggccctgcctgctcctatcgaaaagaccatctccaaggccaagggccagcctagggaaccccaggtttacaccttgcctccatctcgggacgagctgaccaagaaccaggtgtccctgacctgtctcgtgaagggcttctacccctccgatatcgccgtggaatgggagtctaatggccagcctgagaacaactacaagacaacccctcctgtgctggactccgacggctcattcttcctgtactccaagctgacagtggacaagtccagatggcagcagggcaacgtgttctcctgctccgtgatgcacgaggccctgcacaatcactacacccagaagtccctgtctctgtcccctggcaaa

SEQ ID NO: 23 - protein, 447 aa, Homo sapiens
QVELVESGGGLVQPGGSLRLSCAASGFTFSLFTMSWVRQAPGKGLEWVSAISGSGGSTYYADSVKGRFTISRDNSKNTLYLQMNSLRAEDTAVYYCARSTHLYLFDYWGQGTLVTVSSASTKGPSVFPLAPSSKSTSGGTAALGCLVKDYFPEPVTVSWNSGALTSGVHTFPAVLQSSGLYSLSSVVTVPSSSLGTQTYICNVNHKPSNTKVDKKVEPKSCDKTHTCPPCPAPEAAGGPSVFLFPPKPKDTLMISRTPEVTCVVVDVSHEDPEVKFNWYVDGVEVHNAKTKPREQYNSTYRVVSVLTVLHQDWLNGKEYKCKVSNKALPAPIEKTISKAKGQPREPQVYTLPPSRDELTKNQVSLTCLVKGFYPSDIAVEWESNGQPENNYKTTPPVLDSDGSFFLYSKLTVDKSRWQQGNVFSCSVMHEALHNHYTQKSLSLSPGK

SEQ ID NO: 24 - DNA, 1341 bp, Homo sapiens
  source 1..1341: mol_type = other DNA
caggtggaactggtggaatctggcggaggattggttcagcctggcggctctctgagactgtcttgtgccgcctctggcttcaccttcagcctgttcaccatgtcctgggtccgacaggctcctggcaaaggactggaatgggtgtccgccatctctggctctggcggcagcacctactacgccgattctgtgaagggcagattcaccatcagccgggacaactccaagaacaccctgtacctgcagatgaactccctgagagccgaggacaccgccgtgtactactgtgccagaagcacccacctgtatctgttcgactattggggccagggcaccctggtcacagtctcttctgcttctaccaagggacccagcgtgttccctctggctcctagctctaagtccacctctggcggaacagctgctctgggctgtctggtcaaggactacttccctgagcctgtgaccgtgtcttggaactctggcgctctgacatccggcgtgcacacctttccagctgtgctgcaatcctccggcctgtactctctgtcctccgtcgtgaccgtgccttctagctctctgggcacccagacctacatctgcaatgtgaaccacaagccttccaacaccaaggtggacaagaaggtggaacccaagtcctgcgacaagacccacacctgtcctccatgtcctgctccagaagctgctggcggcccttccgtgtttctgttccctccaaagcctaaggacaccctgatgatctctcggacccctgaagtgacctgcgtggtggtggatgtgtctcacgaggacccagaagtgaagttcaattggtacgtggacggcgtggaagtgcacaacgccaagaccaagcctagagagcagtacaactccacctacagagtggtgtccgtgctgaccgtgctgcaccaggattggctgaacggcaaagagtacaagtgcaaggtgtccaacaaggccctgcctgctcctatcgaaaagaccatctccaaggccaagggccagcctagggaaccccaggtttacaccttgcctccatctcgggacgagctgaccaagaaccaggtgtccctgacctgtctcgtgaagggcttctacccctccgatatcgccgtggaatgggagtctaatggccagccagagaacaactacaagacaacccctcctgtgctggactccgacggctcattcttcctgtactccaagctgacagtggacaagtccagatggcagcagggcaacgtgttctcctgctccgtgatgcacgaggccctgcacaatcactacacacagaagtccctgtctctgtcccctggcaag